European Patent Application EP 4 692 307 A1, published February 11, 2026. Title: Kluyveromyces marxianus and Use thereof. Applicant: Angel Yeast Co., Ltd. The sequence listing filed with the application follows.

SEQUENCE LISTING (3 sequences)

SEQ ID NO: 1 - DNA, 19 bp, synthetic construct
  source 1..19: mol_type = other DNA; note = synthetic DNA used as primer
tccgtaggtgaacctgcgg

SEQ ID NO: 2 - DNA, 20 bp, synthetic construct
  source 1..20: mol_type = other DNA; note = synthetic DNA used as primer
tcctccgcttattgatatgc

SEQ ID NO: 3 - DNA, 562 bp, Kluyveromyces marxianus
  source 1..562: mol_type = genomic DNA
ccaacggggattgccttagtacggcgagtgaagcggcaaaagctcaaatttgaaatctggcgtcttcgacgtccgagttgtaatttgaagaaggcgactttgtagctggtccttgtctatgttccttggaacaggacgtcatagagggtgagaatcccgtgtggcgaggatcccagttatttgtaaagtgctttcgacgagtcgagttgtttgggaatgcagctctaagtgggtggtaaattccatctaaagctaaatattggcgagagaccgatagcgaacaagtacagtgatggaaagatgaaaagaactttgaaaagagagtgaaaaagtacgtgaaattgttgaaagggaagggcatttgatcagacatggcgtttgcttcggctttcgctgggccagcatcagttttagcggttggataaatcctcgggaatgtggctctgcttcggtagagtgttatagcccgtgggaatacagccagctgggactgaggattgcgacttttgtcaaggatgctggcgtaatggttaaatgccgcccgtcttgaacccacggacca